European Patent Application EP 4 286 405 A1, published December 6, 2023. Title: GENE THERAPIES FOR TREATING NEURODEGENERATIVE DISORDER. Applicant: ABrain. The sequence listing filed with the application follows.

SEQUENCE LISTING (24 sequences)

SEQ ID NO: 1 - protein, 770 aa, Artificial Sequence
  amyloid precursor protein
MLPGLALLLLAAWTARALEVPTDGNAGLLAEPQIAMFCGRLNMHMNVQNGKWDSDPSGTKTCIDTKEGILQYCQEVYPELQITNVVEANQPVTIQNWCKRGRKQCKTHPHFVIPYRCLVGEFVSDALLVPDKCKFLHQERMDVCETHLHWHTVAKETCSEKSTNLHDYGMLLPCGIDKFRGVEFVCCPLAEESDNVDSADAEEDDSDVWWGGADTDYADGSEDKVVEVAEEEEVAEVEEEEADDDEDDEDGDEVEEEAEEPYEEATERTTSIATTTTTTTESVEEVVREVCSEQAETGPCRAMISRWYFDVTEGKCAPFFYGGCGGNRNNFDTEEYCMAVCGSAMSQSLLKTTQEPLARDPVKLPTTAASTPDAVDKYLETPGDENEHAHFQKAKERLEAKHRERMSQVMREWEEAERQAKNLPKADKKAVIQHFQEKVESLEQEAANERQQLVETHMARVEAMLNDRRRLALENYITALQAVPPRPRHVFNMLKKYVRAEQKDRQHTLKHFEHVRMVDPKKAAQIRSQVMTHLRVIYERMNQSLSLLYNVPAVAEEIQDEVDELLQKEQNYSDDVLANMISEPRISYGNDALMPSLTETKTTVELLPVNGEFSLDDLQPWHSFGADSVPANTENEVEPVDARPAADRGLTTRPGSGLTNIKTEEISEVKMDAEFRHDSGYEVHHQKLVFFAEDVGSNKGAIIGLMVGGVVIATVIVITLVMLKKKQYTSIHHGVVEVDAAVTPEERHLSKMQQNGYENPTYKFFEQMQN

SEQ ID NO: 2 - DNA, 2313 bp, Artificial Sequence
  amyloid precursor protein
atgctgcccggtttggcactgctcctgctggccgcctggacggctcgggcgctggaggtacccactgatggtaatgctggcctgctggctgaaccccagattgccatgttctgtggcagactgaacatgcacatgaatgtccagaatgggaagtgggattcagatccatcagggaccaaaacctgcattgataccaaggaaggcatcctgcagtattgccaagaagtctaccctgaactgcagatcaccaatgtggtagaagccaaccaaccagtgaccatccagaactggtgcaagcggggccgcaagcagtgcaagacccatccccactttgtgattccctaccgctgcttagttggtgagtttgtaagtgatgcccttctcgttcctgacaagtgcaaattcttacaccaggagaggatggatgtttgcgaaactcatcttcactggcacaccgtcgccaaagagacatgcagtgagaagagtaccaacttgcatgactacggcatgttgctgccctgcggaattgacaagttccgaggggtagagtttgtgtgttgcccactggctgaagaaagtgacaatgtggattctgctgatgcggaggaggatgactcggatgtctggtggggcggagcagacacagactatgcagatgggagtgaagacaaagtagtagaagtagcagaggaggaagaagtggctgaggtggaagaagaagaagccgatgatgacgaggacgatgaggatggtgatgaggtagaggaagaggctgaggaaccctacgaagaagccacagagagaaccaccagcattgccaccaccaccaccaccaccacagagtctgtggaagaggtggttcgagaggtgtgctctgaacaagccgagacggggccgtgccgagcaatgatctcccgctggtactttgatgtgactgaagggaagtgtgccccattcttttacggcggatgtggcggcaaccggaacaactttgacacagaagagtactgcatggccgtgtgtggcagcgccatgtcccaaagtttactcaagactacccaggaacctcttgcccgagatcctgttaaacttcctacaacagcagccagtacccctgatgccgttgacaagtatctcgagacacctggggatgagaatgaacatgcccatttccagaaagccaaagagaggcttgaggccaagcaccgagagagaatgtcccaggtcatgagagaatgggaagaggcagaacgtcaagcaaagaacttgcctaaagctgataagaaggcagttatccagcatttccaggagaaagtggaatctttggaacaggaagcagccaacgagagacagcagctggtggagacacacatggccagagtggaagccatgctcaatgaccgccgccgcctggccctggagaactacatcaccgctctgcaggctgttcctcctcggcctcgtcacgtgttcaatatgctaaagaagtatgtccgcgcagaacagaaggacagacagcacaccctaaagcatttcgagcatgtgcgcatggtggatcccaagaaagccgctcagatccggtcccaggttatgacacacctccgtgtgatttatgagcgcatgaatcagtctctctccctgctctacaacgtgcctgcagtggccgaggagattcaggatgaagttgatgagctgcttcagaaagagcaaaactattcagatgacgtcttggccaacatgattagtgaaccaaggatcagttacggaaacgatgctctcatgccatctttgaccgaaacgaaaaccaccgtggagctccttcccgtgaatggagagttcagcctggacgatctccagccgtggcattcttttggggctgactctgtgccagccaacacagaaaacgaagttgagcctgttgatgcccgccctgctgccgaccgaggactgaccactcgaccaggttctgggttgacaaatatcaagacggaggagatctctgaagtgaagatggatgcagaattccgacatgactcaggatatgaagttcatcatcaaaaattggtgttctttgcagaagatgtgggttcaaacaaaggtgcaatcattggactcatggtgggcggtgttgtcatagcgacagtgatcgtcatcaccttggtgatgctgaagaagaaacagtacacatccattcatcatggtgtggtggaggttgacgccgctgtcaccccagaggagcgccacctgtccaagatgcagcagaacggctacgaaaatccaacctacaagttctttgagcagatgcagaactag

SEQ ID NO: 3 - DNA, 2313 bp, Artificial Sequence
  amyloid precursor protein  V689P/A692D
atgctgcccggtttggcactgctcctgctggccgcctggacggctcgggcgctggaggtacccactgatggtaatgctggcctgctggctgaaccccagattgccatgttctgtggcagactgaacatgcacatgaatgtccagaatgggaagtgggattcagatccatcagggaccaaaacctgcattgataccaaggaaggcatcctgcagtattgccaagaagtctaccctgaactgcagatcaccaatgtggtagaagccaaccaaccagtgaccatccagaactggtgcaagcggggccgcaagcagtgcaagacccatccccactttgtgattccctaccgctgcttagttggtgagtttgtaagtgatgcccttctcgttcctgacaagtgcaaattcttacaccaggagaggatggatgtttgcgaaactcatcttcactggcacaccgtcgccaaagagacatgcagtgagaagagtaccaacttgcatgactacggcatgttgctgccctgcggaattgacaagttccgaggggtagagtttgtgtgttgcccactggctgaagaaagtgacaatgtggattctgctgatgcggaggaggatgactcggatgtctggtggggcggagcagacacagactatgcagatgggagtgaagacaaagtagtagaagtagcagaggaggaagaagtggctgaggtggaagaagaagaagccgatgatgacgaggacgatgaggatggtgatgaggtagaggaagaggctgaggaaccctacgaagaagccacagagagaaccaccagcattgccaccaccaccaccaccaccacagagtctgtggaagaggtggttcgagaggtgtgctctgaacaagccgagacggggccgtgccgagcaatgatctcccgctggtactttgatgtgactgaagggaagtgtgccccattcttttacggcggatgtggcggcaaccggaacaactttgacacagaagagtactgcatggccgtgtgtggcagcgccatgtcccaaagtttactcaagactacccaggaacctcttgcccgagatcctgttaaacttcctacaacagcagccagtacccctgatgccgttgacaagtatctcgagacacctggggatgagaatgaacatgcccatttccagaaagccaaagagaggcttgaggccaagcaccgagagagaatgtcccaggtcatgagagaatgggaagaggcagaacgtcaagcaaagaacttgcctaaagctgataagaaggcagttatccagcatttccaggagaaagtggaatctttggaacaggaagcagccaacgagagacagcagctggtggagacacacatggccagagtggaagccatgctcaatgaccgccgccgcctggccctggagaactacatcaccgctctgcaggctgttcctcctcggcctcgtcacgtgttcaatatgctaaagaagtatgtccgcgcagaacagaaggacagacagcacaccctaaagcatttcgagcatgtgcgcatggtggatcccaagaaagccgctcagatccggtcccaggttatgacacacctccgtgtgatttatgagcgcatgaatcagtctctctccctgctctacaacgtgcctgcagtggccgaggagattcaggatgaagttgatgagctgcttcagaaagagcaaaactattcagatgacgtcttggccaacatgattagtgaaccaaggatcagttacggaaacgatgctctcatgccatctttgaccgaaacgaaaaccaccgtggagctccttcccgtgaatggagagttcagcctggacgatctccagccgtggcattcttttggggctgactctgtgccagccaacacagaaaacgaagttgagcctgttgatgcccgccctgctgccgaccgaggactgaccactcgaccaggttctgggttgacaaatatcaagacggaggagatctctgaagtgaagatggatgcagaattccgacatgactcaggatatgaagttcatcatcaaaaattgccgttctttgacgaagatgtgggttcaaacaaaggtgcaatcattggactcatggtgggcggtgttgtcatagcgacagtgatcgtcatcaccttggtgatgctgaagaagaaacagtacacatccattcatcatggtgtggtggaggttgacgccgctgtcaccccagaggagcgccacctgtccaagatgcagcagaacggctacgaaaatccaacctacaagttctttgagcagatgcagaactag

SEQ ID NO: 4 - DNA, 2313 bp, Artificial Sequence
  amyloid precursor protein  V689P/F690D/A692D
atgctgcccggtttggcactgctcctgctggccgcctggacggctcgggcgctggaggtacccactgatggtaatgctggcctgctggctgaaccccagattgccatgttctgtggcagactgaacatgcacatgaatgtccagaatgggaagtgggattcagatccatcagggaccaaaacctgcattgataccaaggaaggcatcctgcagtattgccaagaagtctaccctgaactgcagatcaccaatgtggtagaagccaaccaaccagtgaccatccagaactggtgcaagcggggccgcaagcagtgcaagacccatccccactttgtgattccctaccgctgcttagttggtgagtttgtaagtgatgcccttctcgttcctgacaagtgcaaattcttacaccaggagaggatggatgtttgcgaaactcatcttcactggcacaccgtcgccaaagagacatgcagtgagaagagtaccaacttgcatgactacggcatgttgctgccctgcggaattgacaagttccgaggggtagagtttgtgtgttgcccactggctgaagaaagtgacaatgtggattctgctgatgcggaggaggatgactcggatgtctggtggggcggagcagacacagactatgcagatgggagtgaagacaaagtagtagaagtagcagaggaggaagaagtggctgaggtggaagaagaagaagccgatgatgacgaggacgatgaggatggtgatgaggtagaggaagaggctgaggaaccctacgaagaagccacagagagaaccaccagcattgccaccaccaccaccaccaccacagagtctgtggaagaggtggttcgagaggtgtgctctgaacaagccgagacggggccgtgccgagcaatgatctcccgctggtactttgatgtgactgaagggaagtgtgccccattcttttacggcggatgtggcggcaaccggaacaactttgacacagaagagtactgcatggccgtgtgtggcagcgccatgtcccaaagtttactcaagactacccaggaacctcttgcccgagatcctgttaaacttcctacaacagcagccagtacccctgatgccgttgacaagtatctcgagacacctggggatgagaatgaacatgcccatttccagaaagccaaagagaggcttgaggccaagcaccgagagagaatgtcccaggtcatgagagaatgggaagaggcagaacgtcaagcaaagaacttgcctaaagctgataagaaggcagttatccagcatttccaggagaaagtggaatctttggaacaggaagcagccaacgagagacagcagctggtggagacacacatggccagagtggaagccatgctcaatgaccgccgccgcctggccctggagaactacatcaccgctctgcaggctgttcctcctcggcctcgtcacgtgttcaatatgctaaagaagtatgtccgcgcagaacagaaggacagacagcacaccctaaagcatttcgagcatgtgcgcatggtggatcccaagaaagccgctcagatccggtcccaggttatgacacacctccgtgtgatttatgagcgcatgaatcagtctctctccctgctctacaacgtgcctgcagtggccgaggagattcaggatgaagttgatgagctgcttcagaaagagcaaaactattcagatgacgtcttggccaacatgattagtgaaccaaggatcagttacggaaacgatgctctcatgccatctttgaccgaaacgaaaaccaccgtggagctccttcccgtgaatggagagttcagcctggacgatctccagccgtggcattcttttggggctgactctgtgccagccaacacagaaaacgaagttgagcctgttgatgcccgccctgctgccgaccgaggactgaccactcgaccaggttctgggttgacaaatatcaagacggaggagatctctgaagtgaagatggatgcagaattccgacatgactcaggatatgaagttcatcatcaaaaattgccggactttgacgaagatgtgggttcaaacaaaggtgcaatcattggactcatggtgggcggtgttgtcatagcgacagtgatcgtcatcaccttggtgatgctgaagaagaaacagtacacatccattcatcatggtgtggtggaggttgacgccgctgtcaccccagaggagcgccacctgtccaagatgcagcagaacggctacgaaaatccaacctacaagttctttgagcagatgcagaactag

SEQ ID NO: 5 - protein, 770 aa, Artificial Sequence
  amyloid precursor protein  V689P/A692D
MLPGLALLLLAAWTARALEVPTDGNAGLLAEPQIAMFCGRLNMHMNVQNGKWDSDPSGTKTCIDTKEGILQYCQEVYPELQITNVVEANQPVTIQNWCKRGRKQCKTHPHFVIPYRCLVGEFVSDALLVPDKCKFLHQERMDVCETHLHWHTVAKETCSEKSTNLHDYGMLLPCGIDKFRGVEFVCCPLAEESDNVDSADAEEDDSDVWWGGADTDYADGSEDKVVEVAEEEEVAEVEEEEADDDEDDEDGDEVEEEAEEPYEEATERTTSIATTTTTTTESVEEVVREVCSEQAETGPCRAMISRWYFDVTEGKCAPFFYGGCGGNRNNFDTEEYCMAVCGSAMSQSLLKTTQEPLARDPVKLPTTAASTPDAVDKYLETPGDENEHAHFQKAKERLEAKHRERMSQVMREWEEAERQAKNLPKADKKAVIQHFQEKVESLEQEAANERQQLVETHMARVEAMLNDRRRLALENYITALQAVPPRPRHVFNMLKKYVRAEQKDRQHTLKHFEHVRMVDPKKAAQIRSQVMTHLRVIYERMNQSLSLLYNVPAVAEEIQDEVDELLQKEQNYSDDVLANMISEPRISYGNDALMPSLTETKTTVELLPVNGEFSLDDLQPWHSFGADSVPANTENEVEPVDARPAADRGLTTRPGSGLTNIKTEEISEVKMDAEFRHDSGYEVHHQKLPFFDEDVGSNKGAIIGLMVGGVVIATVIVITLVMLKKKQYTSIHHGVVEVDAAVTPEERHLSKMQQNGYENPTYKFFEQMQN

SEQ ID NO: 6 - protein, 770 aa, Artificial Sequence
  amyloid precursor protein  V689P/F690D/A692D
MLPGLALLLLAAWTARALEVPTDGNAGLLAEPQIAMFCGRLNMHMNVQNGKWDSDPSGTKTCIDTKEGILQYCQEVYPELQITNVVEANQPVTIQNWCKRGRKQCKTHPHFVIPYRCLVGEFVSDALLVPDKCKFLHQERMDVCETHLHWHTVAKETCSEKSTNLHDYGMLLPCGIDKFRGVEFVCCPLAEESDNVDSADAEEDDSDVWWGGADTDYADGSEDKVVEVAEEEEVAEVEEEEADDDEDDEDGDEVEEEAEEPYEEATERTTSIATTTTTTTESVEEVVREVCSEQAETGPCRAMISRWYFDVTEGKCAPFFYGGCGGNRNNFDTEEYCMAVCGSAMSQSLLKTTQEPLARDPVKLPTTAASTPDAVDKYLETPGDENEHAHFQKAKERLEAKHRERMSQVMREWEEAERQAKNLPKADKKAVIQHFQEKVESLEQEAANERQQLVETHMARVEAMLNDRRRLALENYITALQAVPPRPRHVFNMLKKYVRAEQKDRQHTLKHFEHVRMVDPKKAAQIRSQVMTHLRVIYERMNQSLSLLYNVPAVAEEIQDEVDELLQKEQNYSDDVLANMISEPRISYGNDALMPSLTETKTTVELLPVNGEFSLDDLQPWHSFGADSVPANTENEVEPVDARPAADRGLTTRPGSGLTNIKTEEISEVKMDAEFRHDSGYEVHHQKLPDFDEDVGSNKGAIIGLMVGGVVIATVIVITLVMLKKKQYTSIHHGVVEVDAAVTPEERHLSKMQQNGYENPTYKFFEQMQN

SEQ ID NO: 7 - protein, 42 aa, Artificial Sequence [sequence omitted]

SEQ ID NO: 8 - DNA, 126 bp, Artificial Sequence
  Amyloid beta 42
gatgcagaattccgacatgactcaggatatgaagttcatcatcaaaaattggtgttctttgcagaagatgtgggttcaaacaaaggtgcaatcattggactcatggtgggcggtgttgtcatagcg

SEQ ID NO: 9 - DNA, 126 bp, Artificial Sequence
  Amyloid beta 42 (V18P/A21D)
gatgcagaattccgacatgactcaggatatgaagttcatcatcaaaaattgccgttctttgacgaagatgtgggttcaaacaaaggtgcaatcattggactcatggtgggcggtgttgtcatagcg

SEQ ID NO: 10 - DNA, 126 bp, Artificial Sequence
  Amyloid beta 42 (V18P/F19D/A21D)
gatgcagaattccgacatgactcaggatatgaagttcatcatcaaaaattgccggactttgacgaagatgtgggttcaaacaaaggtgcaatcattggactcatggtgggcggtgttgtcatagcg

SEQ ID NO: 11 - protein, 42 aa, Artificial Sequence
  Amyloid beta 42(V18P/A21D)
DAEFRHDSGYEVHHQKLPFFDEDVGSNKGAIIGLMVGGVVIA

SEQ ID NO: 12 - protein, 42 aa, Artificial Sequence
  Amyloid beta 42 (V18P/F19D/A21D)
DAEFRHDSGYEVHHQKLPDFDEDVGSNKGAIIGLMVGGVVIA

SEQ ID NO: 13 - protein, 12 aa, Artificial Sequence
  KK
TVIVITLVMLKK

SEQ ID NO: 14 - DNA, 36 bp, Artificial Sequence
  KK
acagtgatcgtcatcaccttggtgatgctgaagaag

SEQ ID NO: 15 - protein, 23 aa, Artificial Sequence
  gamma secretase cleavage
AIIGLMVGGVVIATVIVITLVML

SEQ ID NO: 16 - DNA, 69 bp, Artificial Sequence
  gamma secretase cleavage
gcaatcattggactcatggtgggcggtgttgtcatagcgacagtgatcgtcatcaccttggtgatgctg

SEQ ID NO: 17 - DNA, 271 bp, Artificial Sequence
  human synapsin I (SYN) promoter
gcggacagtgccttcgcccccgcctggcggcgcgcgccaccgccgcctcagcactgaaggcgcgctgacgtcactcgccggtcccccgcaaactccccttcccggccaccttggtcgcgtccgcgccgccgccggcccagccggaccgcaccacgcgaggcgcgagataggggggcacgggcgcgaccatctgcgctgcggcgccggcgactcagcgctgcctcagtctgcggtgggcagcggaggagtcgtgtcgtgcctgagagcgcag

SEQ ID NO: 18 - DNA, 1293 bp, Artificial Sequence
  CamKII promoter
ttaacattatggccttaggtcacttcatctccatggggttcttcttctgattttctagaaaatgagatgggggtgcagagagcttcctcagtgacctgcccagggtcacatcagaaatgtcagagctagaacttgaactcagattactaatcttaaattccatgccttgggggcatgcaagtacgatatacagaaggagtgaactcattagggcagatgaccaatgagtttaggaaagaagagtccagggcagggtacatctacaccacccgcccagccctgggtgagtccagccacgttcacctcattatagttgcctctctccagtcctaccttgacgggaagcacaagcagaaactgggacaggagccccaggagaccaaatcttcatggtccctctgggaggatgggtggggagagctgtggcagaggcctcaggaggggccctgctgctcagtggtgacagataggggtgagaaagcagacagagtcattccgtcagcattctgggtctgtttggtacttcttctcacgctaaggtggcggtgtgatatgcacaatggctaaaaagcagggagagctggaaagaaacaaggacagagacagaggccaagtcaaccagaccaattcccagaggaagcaaagaaaccattacagagactacaagggggaagggaaggagagatgaattagcttcccctgtaaaccttagaacccagctgttgccagggcaacggggcaatacctgtctcttcagaggagatgaagttgccagggtaactacatcctgtctttctcaaggaccatcccagaatgtggcacccactagccgttaccatagcaactgcctctttgccccacttaatcccatcccgtctgttaaaagggccctatagttggaggtgggggaggtaggaagagcgatgatcacttgtggactaagtttgttcgcatccccttctccaaccccctcagtacatcaccctgggggaacagggtccacttgctcctgggcccacacagtcctgcagtattgtgtatataaggccagggcaaagaggagcaggttttaaagtgaaaggcaggcaggtgttggggaggcagttaccggggcaacgggaacagggcgtttcggaggtggttgccatggggacctggatgctgacgaaggctcgcgaggctgtgagcagccacagtgccctgctcagaagccccaagctcgtcagtcaagccggttctccgtttgcactcaggagcacgggcaggcgagtggcccctagttctgggggcagc

SEQ ID NO: 19 - DNA, 1104 bp, Artificial Sequence
  Tuba1a promoter
tccccctcaaaaaaaaggagcgctggagaaatacaagcccacacaaagagctcgtttttaaactcactcctttctccttacagtttctgaattccgtattagaagggatggctcatttctagggacaaaataacacaggctctggggtgaggtagggtcgggtaagggggcgagcggggaggggtgatgggagagcactaccgctaaagaaagcaagctctctagtaaagcgttaagtactactttgtatattgtttctcttttttcctttctctctctctctctctttgtttgtttttggtttttgagacaggatatcacactatatatccaggccgggtacaaaataaccgcagtcctccgcttcccaatgctgggatttacaggcataaaccactaagggcggttatgatgaccttgagctgcaagtcttcctgcctctgcctcccaggtgctgttgagggtcataggcgtggtctattcatactgagcttctgaattttgctcaaatattaataataatagtaataataataataaccacaataatacaactgtaaaactaaacatttacccacgcctttttgaccatcattcccatagctcttgctactttatttaaagcgaacagagatgttgaatcctgacggaacgtatttaaatttagtgtagtataaatgaaaagctggaatttaccataaagaatctcaacacaaattctgtgattaagtgttggggaaaaccttaaattatcctaactacagtttaaggtttaagctccgtataatcacccaacccccgttttctttcttccctctctacccctccccagctccaccccataatggatgctcggctagttgcttttgcgaggcctttgtctgaaggatgcaaaatctacggatgctagcgagggggggaaggggggagagattacctcataccatgtcgcttgcaccaatcaccactctcctgtcgcggcttctctgggcagacggaggggtctggaccaacaggaaaaggccttggcccatccccatggtgaccgagctgtatataaggaggcgcatccgcccaagtgccgcaggttctcttacatcgacc

SEQ ID NO: 20 - DNA, 1800 bp, Artificial Sequence
  NSE promoter
agagttttggaaagaagaacattacaagactgagctttttattcaagctggggggctcaatccatccttagctctgggttccttactgaaggaagcactcccaccccacagtaccccactcttagctctgagctcctcctctgctcgcccaatccttccaaccccctatggtggtatggctgacacagaaaatgtctgctcctgtatgggacatttgcccctcttctccaaatataagacaggatgaggcctagcttttgctgctccaaagttttaaaagaacacattgcacggcatttagggactctaaagggtggaggaggaatgagggaattgcatcatgccaaggctggtcctcatccatcactgcttccagggcccagagtggcttccaggaggtattcttacaaaggaagcccgatctgtagctaacactcagagcccattttcctgcgttaacccctcccgacctcatatacaggagtaacatgatcagtgacctgggggagctggccaaactgcgggacctgcccaagctgagggccttggtgctgctggacaacccctgtgccgatgagactgactaccgccaggaggccctggtgcagatggcacacctagagcgcctagacaaagagtactatgaggacgaggaccgggcagaagctgaggagatccgacagaggctgaaggaggaacaggagcaagaactcgacccggaccaagacatggaaccgtacctcccgccaacttagtggcacctctagcctgcagggacagtaaaggtgatggcaggaaggcagcccccggaggtcaaaggctgggcacgcgggaggagaggccagagtcagaggctgcgggtatctcagatatgaaggaaagatgagagaggctcaggaagaggtaagaaaagacacaagagaccagagaagggagaagaattagagagggaggcagaggaccgctgtctctacagacatagctggtagagactgggaggaagggatgaaccctgagcgcatgaagggaaggaggtggctggtggtatatggaggatgtagctgggccagggaaaagatcctgcactaaaaatctgaagctaaaaataacaggacacggggtggagaggcgaaaggagggcagagtgaggcagagagactgagaggcctggggatgtgggcattccggtagggcacacagttcacttgtcttctctttttccaggaggccaaagatgctgacctcaagaactcataataccccagtggggaccaccgcattcatagccctgttacaagaagtgggagatgttcctttttgtcccagactggaaatccgttacatcccgaggctcaggttctgtggtggtcatctctgtgtggcttgttctgtgggcctacctaaagtcctaagcacagctctcaagcagatccgaggcgactaagatgctagtaggggttgtctggagagaagagccgaggaggtgggctgtgatggatcagttcagctttcaaataaaaaggcgtttttatattctgtgtcgagttcgtgaacccctgtggtgggcttctccatctgtctgggttagtacctgccactatactggaataaggggacgcctgcttccctcgagttggctggacaaggttatgagcatccgtgtacttatggggttgccagcttggtcctggatcgcccgggcccttcccccacccgttcggttccccaccaccacccgcgctcgtacgtgcgtctccgcctgcagctcttgactcatcggggccccccgggtcacatgcg

SEQ ID NO: 21 - DNA, 1000 bp, Artificial Sequence
  PDGFB Promoter
gcctgcgtgtcccgaggggggtgctgggcccagtgtgagtacgtgtgactgtgactgagacagtgtgactgctgaaggcagggacacagcagctccctgactgggggcagaaggcgttaactgtgtgaaggctggttgtgggtgggtgggctctgggcctcgaacccgggggctgagggagatagtaaacagcagggtgactgacgggaagatcatgttggtagccctgcgaagatgctgcagggctgtgggggtttgtgtgactttgcagttcaacaaattcaaattcagccaacgctggcagggcctgttgtgccaggcaaccagctaggaggaggagactcggacccagcttgcagctgaagggcgctggctgccgggttctgtgggttcaccttgcggtgtcttcccttgctaacactgagtccttacaatagccccatctccaggttgaggctagatggaggggacagagggaagtgacttgcccaaggtgacccaagctcccgagtgccagggcaggatctgaattcaggctctcagactgcagagcctgagtccctccctgccatgcctgtgccagggtggaaatgtctggtcctggaggggagcgtggactcctggccttggctctggagacatccccctagaccacgtgggctcctaacctgtccatggtcactgtgctgaggggcgggacggtgggtcacccctagttcttttttccccagggccagattcatggactgaagggttgctcggctctcagagaccccctaagcgccccgccctggccccaagccctcccccagctcccgcgtcccccccctcctggcgctgactccgggccagaagaggaaaggctgtctccacccacctctcgcactctcccttctcctttataaaggccggaacagctgaaagggtggcaacttctcctcctgcagccgggagcggcctgcctgcctccctgcgcacccgcagcctcccccgctgcctc

SEQ ID NO: 22 - DNA, 1178 bp, Artificial Sequence
  EF-1alpha promoter
ggctccggtgcccgtcagtgggcagagcgcacatcgcccacagtccccgagaagttggggggaggggtcggcaattgaaccggtgcctagagaaggtggcgcggggtaaactgggaaagtgatgtcgtgtactggctccgcctttttcccgagggtgggggagaaccgtatataagtgcagtagtcgccgtgaacgttctttttcgcaacgggtttgccgccagaacacaggtaagtgccgtgtgtggttcccgcgggcctggcctctttacgggttatggcccttgcgtgccttgaattacttccactggctgcagtacgtgattcttgatcccgagcttcgggttggaagtgggtgggagagttcgaggccttgcgcttaaggagccccttcgcctcgtgcttgagttgaggcctggcctgggcgctggggccgccgcgtgcgaatctggtggcaccttcgcgcctgtctcgctgctttcgataagtctctagccatttaaaatttttgatgacctgctgcgacgctttttttctggcaagatagtcttgtaaatgcgggccaagatctgcacactggtatttcggtttttggggccgcgggcggcgacggggcccgtgcgtcccagcgcacatgttcggcgaggcggggcctgcgagcgcggccaccgagaatcggacgggggtagtctcaagctggccggcctgctctggtgcctggcctcgcgccgccgtgtatcgccccgccctgggcggcaaggctggcccggtcggcaccagttgcgtgagcggaaagatggccgcttcccggccctgctgcagggagctcaaaatggaggacgcggcgctcgggagagcgggcgggtgagtcacccacacaaaggaaaagggcctttccgtcctcagccgtcgcttcatgtgactccacggagtaccgggcgccgtccaggcacctcgattagttctcgagcttttggagtacgtcgtctttaggttggggggaggggttttatgcgatggagtttccccacactgagtgggtggagactgaagttaggccagcttggcacttgatgtaattctccttggaatttgccctttttgagtttggatcttggttcattctcaagcctcagacagtggttcaaagtttttttcttccatttcaggtgtcgtga

SEQ ID NO: 23 - DNA, 996 bp, Artificial Sequence
  CAG promoter
tgtagttaatgattaacccgccatgctacttatctacgtagccatgctctaggaagagtaccattgacgtcaataatgacgtatgttcccatagtaacgccaatagggactttccattgacgtcaatgggtggagtatttacggtaaactgcccacttggcagtacatcaagtgtatcatatgccaagtacgccccctattgacgtcaatgacggtaaatggcccgcctggcattatgcccagtacatgaccttatgggactttcctacttggcagtacatctacgtattagtcatcgctattaccatggtcgaggtgagccccacgttctgcttcactctccccatctcccccccctccccacccccaattttgtatttatttattttttaattattttgtgcagcgatgggggcggggggggggggggggcgcgcgccaggcggggcggggcggggcgaggggcggggcggggcgaggcggagaggtgcggcggcagccaatcagagcggcgcgctccgaaagtttccttttatggcgaggcggcggcggcggcggccctataaaaagcgaagcgcgcggcgggcgggagtcgctgcgcgctgccttcgccccgtgccccgctccgccgccgcctcgcgccgcccgccccggctctgactgaccgcgttactcccacaggtgagcgggcgggacggcccttctcctccgggctgtaattagcgcttggtttaatgacggcttgtttcttttctgtggctgcgtgaaagccttgaggggctccgggagggccctttgtgcggggggagcggctcggggctgtccgcggggggacggctgccttcgggggggacggggcagggcggggttcggcttctggcgtgtgaccggcggctctagagcctctgctaaccatgttcatgccttcttctttttcctacagctcctgggcaacgtgctggttattgtgctgtctcatcattttggcaaagaatt

SEQ ID NO: 24 - DNA, 508 bp, Artificial Sequence
  CMV promoter
cgttacataacttacggtaaatggcccgcctggctgaccgcccaacgacccccgcccattgacgtcaataatgacgtatgttcccatagtaacgccaatagggactttccattgacgtcaatgggtggagtatttacggtaaactgcccacttggcagtacatcaagtgtatcatatgccaagtacgccccctattgacgtcaatgacggtaaatggcccgcctggcattatgcccagtacatgaccttatgggactttcctacttggcagtacatctacgtattagtcatcgctattaccatggtgatgcggttttggcagtacatcaatgggcgtggatagcggtttgactcacggggatttccaagtctccaccccattgacgtcaatgggagtttgttttggcaccaaaatcaacgggactttccaaaatgtcgtaacaactccgccccattgacgcaaatgggcggtaggcgtgtacggtgggaggtctatataagcagagct